European Patent Application EP 4 567 106 A1, published June 11, 2025. Title: 케톨산 리덕토아이소머라제 변이체 및 이를 이용한 L-발린 생산 방법. Applicant: 씨제이제일제당 주식회사. The sequence listing filed with the application follows.

SEQUENCE LISTING (66 sequences)

SEQ ID NO: 1 - protein, 338 aa, Corynebacterium glutamicum
MAIELLYDADADLSLIQGRKVAIVGYGSQGHAHSQNLRDSGVEVVIGLREGSKSAEKAKEAGFEVKTTAEAAAWADVIMLLAPDTSQAEIFTNDIEPNLNAGDALLFGHGLNIHFDLIKPADDIIVGMVAPKGPGHLVRRQFVDGKGVPCLIAVDQDPTGTAQALTLSYAAAIGGARAGVIPTTFEAETVTDLFGEQAVLCGGTEELVKVGFEVLTEAGYEPEMAYFEVLHELKLIVDLMFEGGISNMNYSVSDTAEFGGYLSGPRVIDADTKSRMKDILTDIQDGTFTKRLIANVENGNTELEGLRASYNNHPIEETGAKLRDLMSWVKVDARAETA

SEQ ID NO: 2 - DNA, 1017 bp, synthetic construct
  source 1..1017: mol_type = other DNA
atggctattgaactgctttatgatgctgacgctgacctctccttgatccagggccgcaaggttgccatcgttggctacggctcccagggccacgcacactcccagaacctccgcgattctggcgttgaggttgtcattggtctgcgcgagggctccaagtccgcagagaaggcaaaggaagcaggcttcgaggtcaagaccaccgctgaggctgcagcttgggctgacgtcatcatgctcctggctccagacacctccgttgcagaaatcttcaccaacgacatcgagccaaacctgaacgcaggcgacgcactgctgttcggccacggcctgaacattcacttcgacctgatcaagccagctgacgacatcatcgttggcatggttgcgccaaagggcccaggccacttggttcgccgtcagttcgttgatggcaagggtgttccttgcctcatcgcagtcgaccaggacccaaccggaaccgcacaggctctgaccctgtcctacgcagcagcaatcggtggcgcacgcgcaggcgttatcccaaccaccttcgaagctgagaccgtcaccgacctcttcggcgagcaggctgttctctgcggtggcaccgaggaactggtcaaggttggcttcgaggttctcaccgaagctggctacgagccagagatggcatacttcgaggttcttcacgagctcaagctcatcgttgacctcatgttcgaaggtggcatcagcaacatgaactactctgtttctgacaccgctgagttcggtggctacctctccggcccacgcgtcatcgatgcagacaccaagtcccgcatgaaggacatcctgaccgatatccaggacggcaccttcaccaagcgcctcatcgcaaacgttgagaacggcaacaccgaacttgagggccttcgtgcttcctacaacaaccacccaatcgaggagaccggcgctaagctccgcgacctcatgagctgggtcaaggttgacgctcgcgcagaaaccgcttaa

SEQ ID NO: 3 - protein, 338 aa, synthetic construct
MAIELLYDADADLSLIQGRKVAIVGYGSQGHAHSQNLRDSGVEVVIGLREGSKSAEKAKEAGFEVKTTAEAAAWADVIMLLAPDTSVAEIFTNDIEPNLNAGDALLFGHGLNIHFDLIKPADDIIVGMVAPKGPGHLVRRQFVDGKGVPCLIAVDQDPTGTAQALTLSYAAAIGGARAGVIPTTFEAETVTDLFGEQAVLCGGTEELVKVGFEVLTEAGYEPEMAYFEVLHELKLIVDLMFEGGISNMNYSVSDTAEFGGYLSGPRVIDADTKSRMKDILTDIQDGTFTKRLIANVENGNTELEGLRASYNNHPIEETGAKLRDLMSWVKVDARAETA

SEQ ID NO: 4 - DNA, 31 bp, synthetic construct
  source 1..31: mol_type = other DNA
cccggggcactgcttgatgtgatggaaccat

SEQ ID NO: 5 - DNA, 29 bp, synthetic construct
  source 1..29: mol_type = other DNA
cccggggtcaacgatgagcttgagctcgt

SEQ ID NO: 6 - DNA, 41 bp, synthetic construct
  source 1..41: mol_type = other DNA
cggggatcccccgggaggacggtactcaaatactaaacttc

SEQ ID NO: 7 - DNA, 38 bp, synthetic construct
  source 1..38: mol_type = other DNA
tgccgagtgtttcggtctttacagacacgagggacacg

SEQ ID NO: 8 - DNA, 31 bp, synthetic construct
  source 1..31: mol_type = other DNA
tgtctgtaaagaccgaaacactcggcatcaa

SEQ ID NO: 9 - DNA, 41 bp, synthetic construct
  source 1..41: mol_type = other DNA
cggggatcccccggggacaactacattattattataccaca

SEQ ID NO: 10 - DNA, 18 bp, synthetic construct
  source 1..18: mol_type = other DNA
ccgcgtcaccaaagcgga

SEQ ID NO: 11 - DNA, 20 bp, synthetic construct
  source 1..20: mol_type = other DNA
ttagatcttggccggagcca

SEQ ID NO: 12 - protein, 338 aa, synthetic construct
MAIELLYDADADLSLIQGRKVAIVGYGSQGHAHSQNLRDSGVEVVIGLREGSKSAEKAKEAGFEVKTTAEAAAWADVIMLLAPDTSAAEIFTNDIEPNLNAGDALLFGHGLNIHFDLIKPADDIIVGMVAPKGPGHLVRRQFVDGKGVPCLIAVDQDPTGTAQALTLSYAAAIGGARAGVIPTTFEAETVTDLFGEQAVLCGGTEELVKVGFEVLTEAGYEPEMAYFEVLHELKLIVDLMFEGGISNMNYSVSDTAEFGGYLSGPRVIDADTKSRMKDILTDIQDGTFTKRLIANVENGNTELEGLRASYNNHPIEETGAKLRDLMSWVKVDARAETA

SEQ ID NO: 13 - protein, 338 aa, synthetic construct
MAIELLYDADADLSLIQGRKVAIVGYGSQGHAHSQNLRDSGVEVVIGLREGSKSAEKAKEAGFEVKTTAEAAAWADVIMLLAPDTSIAEIFTNDIEPNLNAGDALLFGHGLNIHFDLIKPADDIIVGMVAPKGPGHLVRRQFVDGKGVPCLIAVDQDPTGTAQALTLSYAAAIGGARAGVIPTTFEAETVTDLFGEQAVLCGGTEELVKVGFEVLTEAGYEPEMAYFEVLHELKLIVDLMFEGGISNMNYSVSDTAEFGGYLSGPRVIDADTKSRMKDILTDIQDGTFTKRLIANVENGNTELEGLRASYNNHPIEETGAKLRDLMSWVKVDARAETA

SEQ ID NO: 14 - protein, 338 aa, synthetic construct
MAIELLYDADADLSLIQGRKVAIVGYGSQGHAHSQNLRDSGVEVVIGLREGSKSAEKAKEAGFEVKTTAEAAAWADVIMLLAPDTSGAEIFTNDIEPNLNAGDALLFGHGLNIHFDLIKPADDIIVGMVAPKGPGHLVRRQFVDGKGVPCLIAVDQDPTGTAQALTLSYAAAIGGARAGVIPTTFEAETVTDLFGEQAVLCGGTEELVKVGFEVLTEAGYEPEMAYFEVLHELKLIVDLMFEGGISNMNYSVSDTAEFGGYLSGPRVIDADTKSRMKDILTDIQDGTFTKRLIANVENGNTELEGLRASYNNHPIEETGAKLRDLMSWVKVDARAETA

SEQ ID NO: 15 - protein, 338 aa, synthetic construct
MAIELLYDADADLSLIQGRKVAIVGYGSQGHAHSQNLRDSGVEVVIGLREGSKSAEKAKEAGFEVKTTAEAAAWADVIMLLAPDTSFAEIFTNDIEPNLNAGDALLFGHGLNIHFDLIKPADDIIVGMVAPKGPGHLVRRQFVDGKGVPCLIAVDQDPTGTAQALTLSYAAAIGGARAGVIPTTFEAETVTDLFGEQAVLCGGTEELVKVGFEVLTEAGYEPEMAYFEVLHELKLIVDLMFEGGISNMNYSVSDTAEFGGYLSGPRVIDADTKSRMKDILTDIQDGTFTKRLIANVENGNTELEGLRASYNNHPIEETGAKLRDLMSWVKVDARAETA

SEQ ID NO: 16 - protein, 338 aa, synthetic construct
MAIELLYDADADLSLIQGRKVAIVGYGSQGHAHSQNLRDSGVEVVIGLREGSKSAEKAKEAGFEVKTTAEAAAWADVIMLLAPDTSMAEIFTNDIEPNLNAGDALLFGHGLNIHFDLIKPADDIIVGMVAPKGPGHLVRRQFVDGKGVPCLIAVDQDPTGTAQALTLSYAAAIGGARAGVIPTTFEAETVTDLFGEQAVLCGGTEELVKVGFEVLTEAGYEPEMAYFEVLHELKLIVDLMFEGGISNMNYSVSDTAEFGGYLSGPRVIDADTKSRMKDILTDIQDGTFTKRLIANVENGNTELEGLRASYNNHPIEETGAKLRDLMSWVKVDARAETA

SEQ ID NO: 17 - protein, 338 aa, synthetic construct
MAIELLYDADADLSLIQGRKVAIVGYGSQGHAHSQNLRDSGVEVVIGLREGSKSAEKAKEAGFEVKTTAEAAAWADVIMLLAPDTSSAEIFTNDIEPNLNAGDALLFGHGLNIHFDLIKPADDIIVGMVAPKGPGHLVRRQFVDGKGVPCLIAVDQDPTGTAQALTLSYAAAIGGARAGVIPTTFEAETVTDLFGEQAVLCGGTEELVKVGFEVLTEAGYEPEMAYFEVLHELKLIVDLMFEGGISNMNYSVSDTAEFGGYLSGPRVIDADTKSRMKDILTDIQDGTFTKRLIANVENGNTELEGLRASYNNHPIEETGAKLRDLMSWVKVDARAETA

SEQ ID NO: 18 - protein, 338 aa, synthetic construct
MAIELLYDADADLSLIQGRKVAIVGYGSQGHAHSQNLRDSGVEVVIGLREGSKSAEKAKEAGFEVKTTAEAAAWADVIMLLAPDTSPAEIFTNDIEPNLNAGDALLFGHGLNIHFDLIKPADDIIVGMVAPKGPGHLVRRQFVDGKGVPCLIAVDQDPTGTAQALTLSYAAAIGGARAGVIPTTFEAETVTDLFGEQAVLCGGTEELVKVGFEVLTEAGYEPEMAYFEVLHELKLIVDLMFEGGISNMNYSVSDTAEFGGYLSGPRVIDADTKSRMKDILTDIQDGTFTKRLIANVENGNTELEGLRASYNNHPIEETGAKLRDLMSWVKVDARAETA

SEQ ID NO: 19 - protein, 338 aa, synthetic construct
MAIELLYDADADLSLIQGRKVAIVGYGSQGHAHSQNLRDSGVEVVIGLREGSKSAEKAKEAGFEVKTTAEAAAWADVIMLLAPDTSTAEIFTNDIEPNLNAGDALLFGHGLNIHFDLIKPADDIIVGMVAPKGPGHLVRRQFVDGKGVPCLIAVDQDPTGTAQALTLSYAAAIGGARAGVIPTTFEAETVTDLFGEQAVLCGGTEELVKVGFEVLTEAGYEPEMAYFEVLHELKLIVDLMFEGGISNMNYSVSDTAEFGGYLSGPRVIDADTKSRMKDILTDIQDGTFTKRLIANVENGNTELEGLRASYNNHPIEETGAKLRDLMSWVKVDARAETA

SEQ ID NO: 20 - protein, 338 aa, synthetic construct
MAIELLYDADADLSLIQGRKVAIVGYGSQGHAHSQNLRDSGVEVVIGLREGSKSAEKAKEAGFEVKTTAEAAAWADVIMLLAPDTSYAEIFTNDIEPNLNAGDALLFGHGLNIHFDLIKPADDIIVGMVAPKGPGHLVRRQFVDGKGVPCLIAVDQDPTGTAQALTLSYAAAIGGARAGVIPTTFEAETVTDLFGEQAVLCGGTEELVKVGFEVLTEAGYEPEMAYFEVLHELKLIVDLMFEGGISNMNYSVSDTAEFGGYLSGPRVIDADTKSRMKDILTDIQDGTFTKRLIANVENGNTELEGLRASYNNHPIEETGAKLRDLMSWVKVDARAETA

SEQ ID NO: 21 - protein, 338 aa, synthetic construct
MAIELLYDADADLSLIQGRKVAIVGYGSQGHAHSQNLRDSGVEVVIGLREGSKSAEKAKEAGFEVKTTAEAAAWADVIMLLAPDTSHAEIFTNDIEPNLNAGDALLFGHGLNIHFDLIKPADDIIVGMVAPKGPGHLVRRQFVDGKGVPCLIAVDQDPTGTAQALTLSYAAAIGGARAGVIPTTFEAETVTDLFGEQAVLCGGTEELVKVGFEVLTEAGYEPEMAYFEVLHELKLIVDLMFEGGISNMNYSVSDTAEFGGYLSGPRVIDADTKSRMKDILTDIQDGTFTKRLIANVENGNTELEGLRASYNNHPIEETGAKLRDLMSWVKVDARAETA

SEQ ID NO: 22 - protein, 338 aa, synthetic construct; identical to SEQ ID NO: 1

SEQ ID NO: 23 - protein, 338 aa, synthetic construct
MAIELLYDADADLSLIQGRKVAIVGYGSQGHAHSQNLRDSGVEVVIGLREGSKSAEKAKEAGFEVKTTAEAAAWADVIMLLAPDTSNAEIFTNDIEPNLNAGDALLFGHGLNIHFDLIKPADDIIVGMVAPKGPGHLVRRQFVDGKGVPCLIAVDQDPTGTAQALTLSYAAAIGGARAGVIPTTFEAETVTDLFGEQAVLCGGTEELVKVGFEVLTEAGYEPEMAYFEVLHELKLIVDLMFEGGISNMNYSVSDTAEFGGYLSGPRVIDADTKSRMKDILTDIQDGTFTKRLIANVENGNTELEGLRASYNNHPIEETGAKLRDLMSWVKVDARAETA

SEQ ID NO: 24 - protein, 338 aa, synthetic construct
MAIELLYDADADLSLIQGRKVAIVGYGSQGHAHSQNLRDSGVEVVIGLREGSKSAEKAKEAGFEVKTTAEAAAWADVIMLLAPDTSKAEIFTNDIEPNLNAGDALLFGHGLNIHFDLIKPADDIIVGMVAPKGPGHLVRRQFVDGKGVPCLIAVDQDPTGTAQALTLSYAAAIGGARAGVIPTTFEAETVTDLFGEQAVLCGGTEELVKVGFEVLTEAGYEPEMAYFEVLHELKLIVDLMFEGGISNMNYSVSDTAEFGGYLSGPRVIDADTKSRMKDILTDIQDGTFTKRLIANVENGNTELEGLRASYNNHPIEETGAKLRDLMSWVKVDARAETA

SEQ ID NO: 25 - protein, 338 aa, synthetic construct
MAIELLYDADADLSLIQGRKVAIVGYGSQGHAHSQNLRDSGVEVVIGLREGSKSAEKAKEAGFEVKTTAEAAAWADVIMLLAPDTSDAEIFTNDIEPNLNAGDALLFGHGLNIHFDLIKPADDIIVGMVAPKGPGHLVRRQFVDGKGVPCLIAVDQDPTGTAQALTLSYAAAIGGARAGVIPTTFEAETVTDLFGEQAVLCGGTEELVKVGFEVLTEAGYEPEMAYFEVLHELKLIVDLMFEGGISNMNYSVSDTAEFGGYLSGPRVIDADTKSRMKDILTDIQDGTFTKRLIANVENGNTELEGLRASYNNHPIEETGAKLRDLMSWVKVDARAETA

SEQ ID NO: 26 - protein, 338 aa, synthetic construct
MAIELLYDADADLSLIQGRKVAIVGYGSQGHAHSQNLRDSGVEVVIGLREGSKSAEKAKEAGFEVKTTAEAAAWADVIMLLAPDTSCAEIFTNDIEPNLNAGDALLFGHGLNIHFDLIKPADDIIVGMVAPKGPGHLVRRQFVDGKGVPCLIAVDQDPTGTAQALTLSYAAAIGGARAGVIPTTFEAETVTDLFGEQAVLCGGTEELVKVGFEVLTEAGYEPEMAYFEVLHELKLIVDLMFEGGISNMNYSVSDTAEFGGYLSGPRVIDADTKSRMKDILTDIQDGTFTKRLIANVENGNTELEGLRASYNNHPIEETGAKLRDLMSWVKVDARAETA

SEQ ID NO: 27 - protein, 338 aa, synthetic construct
MAIELLYDADADLSLIQGRKVAIVGYGSQGHAHSQNLRDSGVEVVIGLREGSKSAEKAKEAGFEVKTTAEAAAWADVIMLLAPDTSWAEIFTNDIEPNLNAGDALLFGHGLNIHFDLIKPADDIIVGMVAPKGPGHLVRRQFVDGKGVPCLIAVDQDPTGTAQALTLSYAAAIGGARAGVIPTTFEAETVTDLFGEQAVLCGGTEELVKVGFEVLTEAGYEPEMAYFEVLHELKLIVDLMFEGGISNMNYSVSDTAEFGGYLSGPRVIDADTKSRMKDILTDIQDGTFTKRLIANVENGNTELEGLRASYNNHPIEETGAKLRDLMSWVKVDARAETA

SEQ ID NO: 28 - protein, 338 aa, synthetic construct
MAIELLYDADADLSLIQGRKVAIVGYGSQGHAHSQNLRDSGVEVVIGLREGSKSAEKAKEAGFEVKTTAEAAAWADVIMLLAPDTSRAEIFTNDIEPNLNAGDALLFGHGLNIHFDLIKPADDIIVGMVAPKGPGHLVRRQFVDGKGVPCLIAVDQDPTGTAQALTLSYAAAIGGARAGVIPTTFEAETVTDLFGEQAVLCGGTEELVKVGFEVLTEAGYEPEMAYFEVLHELKLIVDLMFEGGISNMNYSVSDTAEFGGYLSGPRVIDADTKSRMKDILTDIQDGTFTKRLIANVENGNTELEGLRASYNNHPIEETGAKLRDLMSWVKVDARAETA

SEQ ID NO: 29 - protein, 338 aa, synthetic construct
MAIELLYDADADLSLIQGRKVAIVGYGSQGHAHSQNLRDSGVEVVIGLREGSKSAEKAKEAGFEVKTTAEAAAWADVIMLLAPDTSEAEIFTNDIEPNLNAGDALLFGHGLNIHFDLIKPADDIIVGMVAPKGPGHLVRRQFVDGKGVPCLIAVDQDPTGTAQALTLSYAAAIGGARAGVIPTTFEAETVTDLFGEQAVLCGGTEELVKVGFEVLTEAGYEPEMAYFEVLHELKLIVDLMFEGGISNMNYSVSDTAEFGGYLSGPRVIDADTKSRMKDILTDIQDGTFTKRLIANVENGNTELEGLRASYNNHPIEETGAKLRDLMSWVKVDARAETA

SEQ ID NO: 30 - DNA, 32 bp, synthetic construct
  source 1..32: mol_type = other DNA
cagacacctccgcggcagaaatcttcaccaac

SEQ ID NO: 31 - DNA, 32 bp, synthetic construct
  source 1..32: mol_type = other DNA
aagatttctgccgcggaggtgtctggagccag

SEQ ID NO: 32 - DNA, 32 bp, synthetic construct
  source 1..32: mol_type = other DNA
cagacacctccattgcagaaatcttcaccaac

SEQ ID NO: 33 - DNA, 32 bp, synthetic construct
  source 1..32: mol_type = other DNA
aagatttctgcaatggaggtgtctggagccag

SEQ ID NO: 34 - DNA, 32 bp, synthetic construct
  source 1..32: mol_type = other DNA
cagacacctccggagcagaaatcttcaccaac

SEQ ID NO: 35 - DNA, 32 bp, synthetic construct
  source 1..32: mol_type = other DNA
aagatttctgctccggaggtgtctggagccag

SEQ ID NO: 36 - DNA, 32 bp, synthetic construct
  source 1..32: mol_type = other DNA
cagacacctccttcgcagaaatcttcaccaac

SEQ ID NO: 37 - DNA, 32 bp, synthetic construct
  source 1..32: mol_type = other DNA
aagatttctgcgaaggaggtgtctggagccag

SEQ ID NO: 38 - DNA, 32 bp, synthetic construct
  source 1..32: mol_type = other DNA
cagacacctccatggcagaaatcttcaccaac

SEQ ID NO: 39 - DNA, 32 bp, synthetic construct
  source 1..32: mol_type = other DNA
aagatttctgccatggaggtgtctggagccag

SEQ ID NO: 40 - DNA, 32 bp, synthetic construct
  source 1..32: mol_type = other DNA
cagacacctcctctgcagaaatcttcaccaac

SEQ ID NO: 41 - DNA, 32 bp, synthetic construct
  source 1..32: mol_type = other DNA
aagatttctgcagaggaggtgtctggagccag

SEQ ID NO: 42 - DNA, 32 bp, synthetic construct
  source 1..32: mol_type = other DNA
cagacacctcccctgcagaaatcttcaccaac

SEQ ID NO: 43 - DNA, 32 bp, synthetic construct
  source 1..32: mol_type = other DNA
aagatttctgcaggggaggtgtctggagccag

SEQ ID NO: 44 - DNA, 32 bp, synthetic construct
  source 1..32: mol_type = other DNA
cagacacctccaccgcagaaatcttcaccaac

SEQ ID NO: 45 - DNA, 32 bp, synthetic construct
  source 1..32: mol_type = other DNA
aagatttctgcggtggaggtgtctggagccag

SEQ ID NO: 46 - DNA, 32 bp, synthetic construct
  source 1..32: mol_type = other DNA
cagacacctcctatgcagaaatcttcaccaac

SEQ ID NO: 47 - DNA, 32 bp, synthetic construct
  source 1..32: mol_type = other DNA
aagatttctgcataggaggtgtctggagccag

SEQ ID NO: 48 - DNA, 32 bp, synthetic construct
  source 1..32: mol_type = other DNA
cagacacctcccatgcagaaatcttcaccaac

SEQ ID NO: 49 - DNA, 32 bp, synthetic construct
  source 1..32: mol_type = other DNA
aagatttctgcatgggaggtgtctggagccag

SEQ ID NO: 50 - DNA, 32 bp, synthetic construct
  source 1..32: mol_type = other DNA
cagacacctcccaggcagaaatcttcaccaac

SEQ ID NO: 51 - DNA, 32 bp, synthetic construct
  source 1..32: mol_type = other DNA
aagatttctgcctgggaggtgtctggagccag

SEQ ID NO: 52 - DNA, 32 bp, synthetic construct
  source 1..32: mol_type = other DNA
cagacacctccaatgcagaaatcttcaccaac

SEQ ID NO: 53 - DNA, 32 bp, synthetic construct
  source 1..32: mol_type = other DNA
aagatttctgcattggaggtgtctggagccag

SEQ ID NO: 54 - DNA, 32 bp, synthetic construct
  source 1..32: mol_type = other DNA
cagacacctccaaggcagaaatcttcaccaac

SEQ ID NO: 55 - DNA, 32 bp, synthetic construct
  source 1..32: mol_type = other DNA
aagatttctgccttggaggtgtctggagccag

SEQ ID NO: 56 - DNA, 32 bp, synthetic construct
  source 1..32: mol_type = other DNA
cagacacctccgatgcagaaatcttcaccaac

SEQ ID NO: 57 - DNA, 32 bp, synthetic construct
  source 1..32: mol_type = other DNA
aagatttctgcatcggaggtgtctggagccag

SEQ ID NO: 58 - DNA, 32 bp, synthetic construct
  source 1..32: mol_type = other DNA
cagacacctcctgtgcagaaatcttcaccaac

SEQ ID NO: 59 - DNA, 32 bp, synthetic construct
  source 1..32: mol_type = other DNA
aagatttctgcacaggaggtgtctggagccag

SEQ ID NO: 60 - DNA, 32 bp, synthetic construct
  source 1..32: mol_type = other DNA
cagacacctcctgggcagaaatcttcaccaac

SEQ ID NO: 61 - DNA, 32 bp, synthetic construct
  source 1..32: mol_type = other DNA
aagatttctgcccaggaggtgtctggagccag

SEQ ID NO: 62 - DNA, 32 bp, synthetic construct
  source 1..32: mol_type = other DNA
cagacacctccagagcagaaatcttcaccaac

SEQ ID NO: 63 - DNA, 32 bp, synthetic construct
  source 1..32: mol_type = other DNA
aagatttctgctctggaggtgtctggagccag

SEQ ID NO: 64 - DNA, 32 bp, synthetic construct
  source 1..32: mol_type = other DNA
cagacacctccgaagcagaaatcttcaccaac

SEQ ID NO: 65 - DNA, 32 bp, synthetic construct
  source 1..32: mol_type = other DNA
aagatttctgcttcggaggtgtctggagccag

SEQ ID NO: 66 - DNA, 1017 bp, Corynebacterium glutamicum
  source 1..1017: mol_type = genomic DNA
atggctattgaactgctttatgatgctgacgctgacctctccttgatccagggccgcaaggttgccatcgttggctacggctcccagggccacgcacactcccagaacctccgcgattctggcgttgaggttgtcattggtctgcgcgagggctccaagtccgcagagaaggcaaaggaagcaggcttcgaggtcaagaccaccgctgaggctgcagcttgggctgacgtcatcatgctcctggctccagacacctcccaggcagaaatcttcaccaacgacatcgagccaaacctgaacgcaggcgacgcactgctgttcggccacggcctgaacattcacttcgacctgatcaagccagctgacgacatcatcgttggcatggttgcgccaaagggcccaggccacttggttcgccgtcagttcgttgatggcaagggtgttccttgcctcatcgcagtcgaccaggacccaaccggaaccgcacaggctctgaccctgtcctacgcagcagcaatcggtggcgcacgcgcaggcgttatcccaaccaccttcgaagctgagaccgtcaccgacctcttcggcgagcaggctgttctctgcggtggcaccgaggaactggtcaaggttggcttcgaggttctcaccgaagctggctacgagccagagatggcatacttcgaggttcttcacgagctcaagctcatcgttgacctcatgttcgaaggtggcatcagcaacatgaactactctgtttctgacaccgctgagttcggtggctacctctccggcccacgcgtcatcgatgcagacaccaagtcccgcatgaaggacatcctgaccgatatccaggacggcaccttcaccaagcgcctcatcgcaaacgttgagaacggcaacaccgaacttgagggccttcgtgcttcctacaacaaccacccaatcgaggagaccggcgctaagctccgcgacctcatgagctgggtcaaggttgacgctcgcgcagaaaccgcttaa